European Patent Application EP 4 810 524 A1, published September 23, 2026. Title: 一种靶向CD38和CLL1的双特异性嵌合抗原受体及其应用. Applicant: 亘喜生物科技（上海）有限公司. The sequence listing filed with the application follows.

SEQUENCE LISTING (51 sequences)

SEQ ID NO: 1 - protein, 116 aa, synthetic construct
QVQLVESGGGLVQAGGSLRLACTASGNIFASQVMNWYRQAPGSPRELVATITPGGRTTYADSAKGRFTVATDNAKATAYLQLTSLTPEDTGVYYCHVRLFPATDYWGQGTQVTVSS

SEQ ID NO: 2 - protein, 126 aa, synthetic construct
QVQLVESGGGLVQPGGSLRLSCTASGFRLDYYAIGWFRQAPGKEREAISCIDITGMHTNYGDSVMGRFTISRDDAKRTVYLQMNSLEAEDTGIYYCAPAQYAACSALGVKVSFTSWGQGTQVTVSP

SEQ ID NO: 3 - protein, 126 aa, synthetic construct
QVQLVESGGGLVQPGGSLRLSCTASGFRLDYYAIGWFRQAPGKEREAIACIDITGFHTNYGDSVSGRFTISRDNAGTTVYLQMNSLEAEDTGIYYCAPARYAACSALDVKLSFTSWGQGTQVTVSS

SEQ ID NO: 4 - protein, 118 aa, synthetic construct
QVQLVESGGGLVQPGGSLRLSCAASGFTFSSYAMGWARQVPGKEVEWVSGIYSDGSTNYADSVKGRFTISRDNAKNTVYLQMNSLRPEDTAVYHCATDPTVHSDLPVWGQGTLVTVSS

SEQ ID NO: 5 - protein, 118 aa, synthetic construct
QVQLVESGGGLVQPGGSLRLSCAASGFTFSSYAMGWARQVPGKDVEWVSGIYSDGSTYYADSVKGRFTISRYNAKNTVYLQMNSLKPEDTAVYYCATDPTLENQTTAWGQGTQVTVSS

SEQ ID NO: 6 - protein, 5 aa, synthetic construct
SQVMN

SEQ ID NO: 7 - protein, 5 aa, synthetic construct
YYAIG

SEQ ID NO: 8 - protein, 16 aa, synthetic construct
TITPGGRTTYADSAKG

SEQ ID NO: 9 - protein, 17 aa, synthetic construct
CIDITGMHTNYGDSVMG

SEQ ID NO: 10 - protein, 17 aa, synthetic construct
CIDITGFHTNYGDSVSG

SEQ ID NO: 11 - protein, 8 aa, synthetic construct
RLFPATDY

SEQ ID NO: 12 - protein, 17 aa, synthetic construct
AQYAACSALGVKVSFTS

SEQ ID NO: 13 - protein, 17 aa, synthetic construct
ARYAACSALDVKLSFTS

SEQ ID NO: 14 - protein, 5 aa, synthetic construct
SYAMG

SEQ ID NO: 15 - protein, 16 aa, synthetic construct
GIYSDGSTNYADSVKG

SEQ ID NO: 16 - protein, 16 aa, synthetic construct
GIYSDGSTYYADSVKG

SEQ ID NO: 17 - protein, 10 aa, synthetic construct
DPTVHSDLPV

SEQ ID NO: 18 - protein, 10 aa, synthetic construct
DPTLENQTTA

SEQ ID NO: 19 - protein, 24 aa, synthetic construct
IYIWAPLAGTCGVLLLSLVITLYC

SEQ ID NO: 20 - protein, 27 aa, synthetic construct
FWVLVVVGGVLACYSLLVTVAFIIFWV

SEQ ID NO: 21 - protein, 112 aa, synthetic construct
RVKFSRSADAPAYQQGQNQLYNELNLGRREEYDVLDKRRGRDPEMGGKPRRKNPQEGLYNELQKDKMAEAYSEIGMKGERRRGKGHDGLYQGLSTATKDTYDALHMQALPPR

SEQ ID NO: 22 - protein, 42 aa, synthetic construct
KRGRKKLLYIFKQPFMRPVQTTQEEDGCSCRFPEEEEGGCEL

SEQ ID NO: 23 - protein, 41 aa, synthetic construct
RSKRSRLLHSDYMNMTPRRPGPTRKHYQPYAPPRDFAAYRS

SEQ ID NO: 24 - protein, 42 aa, synthetic construct
PAPRPPTPAPTIASQPLSLRPEACRPAAGGAVHTRGLDFACD

SEQ ID NO: 25 - protein, 21 aa, synthetic construct
MALPVTALLLPLALLLHAARP

SEQ ID NO: 26 - protein, 15 aa, synthetic construct
GGGGSGGGGSGGGGS

SEQ ID NO: 27 - protein, 8 aa, synthetic construct
DYKDDDDK

SEQ ID NO: 28 - DNA, 1512 bp, synthetic construct
  source 1..1512: mol_type = other DNA
atggccttaccagtgaccgccttgctcctgccgctggccttgctgctccacgccgccaggccgcaagttcagcttgttgaatctggcggcggactggttcagcctggcggatctctgagactgtcttgtgccgccagcggcttcacctttagcagctatgctatgggctgggccagacaggtgccaggcaaagaggttgaatgggtgtccggcatctacagcgacggcagcaccaattacgccgacagcgtgaagggcagattcaccatcagccgggacaacgccaagaacaccgtgtacctgcagatgaacagcctgcggcctgaggatacagccgtgtaccactgtgccaccgatcctaccgtgcacagcgatctgcctgtttggggacagggcacactggtcacagtttctagcggaggcggaggatcaggtggcggtggatctggcggtggtggttctcaggtgcagctggttgaaagcggcggaggacttgtgcaaccaggcggaagcctgagactgagctgtaccgcctctggcttccggctggattactatgccatcggctggttcaggcaggcccctggcaaagagagagaggccatcagctgcatcgacatcaccggcatgcacaccaactacggcgattccgtgatggggcgcttcaccatctccagagatgacgccaagcggacagtgtatctccagatgaattccctggaagccgaggacacaggcatctactactgtgcccctgctcagtacgccgcctgttctgctctgggcgtgaaggtgtcctttacctcttggggccagggaacccaagtgaccgtttctcctacaacgacaccagcaccacggccacccactcctgctccgacaattgcgtctcagcccctttcccttcgacccgaagcttgtcgccctgctgcgggaggagcggtccacacgcgcgggcttgacttcgcttgcgacatctacatttgggcacccttggccgggacatgcggcgtcttgctcctgagtctggttataacgctgtattgtaagcgaggtcggaagaagcttttgtatatctttaaacagccctttatgaggcccgtacaaaccacacaagaggaggatgggtgctcatgcagatttcctgaagaggaagagggcggttgcgaacttagagtcaaattcagccgctccgcagatgcacctgcttataaacagggtcagaatcaattgtataatgaacttaatctcgggaggcgcgaggagtatgatgtgctggacaagcgacggggtcgagacccagagatgggcggtaaaccccgccgaaagaacccccaggagggactgtataatgagctgcaaaaggacaaaatggcagaagcctattccgaaatagggatgaagggagagcggcggcgaggtaagggacatgacggtctttatcaaggtcttagtactgcaactaaggacacctatgacgcgctgcatatgcaggctctcccacctagataa

SEQ ID NO: 29 - DNA, 1512 bp, synthetic construct
  source 1..1512: mol_type = other DNA
atggccttaccagtgaccgccttgctcctgccgctggccttgctgctccacgccgccaggccgcaagttcagcttgttgaatctggcggcggactggttcagcctggcggatctctgagactgtcttgtgccgccagcggcttcacctttagcagctatgctatgggctgggccagacaggtgccaggcaaagaggttgaatgggtgtccggcatctacagcgacggcagcaccaattacgccgacagcgtgaagggcagattcaccatcagccgggacaacgccaagaacaccgtgtacctgcagatgaacagcctgcggcctgaggatacagccgtgtaccactgtgccaccgatcctaccgtgcacagcgatctgcctgtttggggacagggcacactggtcacagtttctagcggaggcggaggatcaggtggcggtggatctggcggtggtggttctcaggtgcagctggttgaaagcggcggaggacttgtgcaaccaggcggaagcctgagactgagctgtaccgcctctggcttccggctggattactatgccatcggctggttcaggcaggcccctggcaaagagagagaggccattgcctgcatcgacatcaccggcttccacaccaactacggcgattccgtgtctggccggttcaccatctccagagataatgccggcaccacagtgtatctccagatgaattccctggaagccgaggacacaggcatctactactgtgcccctgccagatacgccgcctgttctgccctggatgtgaagctgagctttacctcttggggccagggaacccaagtgaccgttagctctacaacgacaccagcaccacggccacccactcctgctccgacaattgcgtctcagcccctttcccttcgacccgaagcttgtcgccctgctgcgggaggagcggtccacacgcgcgggcttgacttcgcttgcgacatctacatttgggcacccttggccgggacatgcggcgtcttgctcctgagtctggttataacgctgtattgtaagcgaggtcggaagaagcttttgtatatctttaaacagccctttatgaggcccgtacaaaccacacaagaggaggatgggtgctcatgcagatttcctgaagaggaagagggcggttgcgaacttagagtcaaattcagccgctccgcagatgcacctgcttataaacagggtcagaatcaattgtataatgaacttaatctcgggaggcgcgaggagtatgatgtgctggacaagcgacggggtcgagacccagagatgggcggtaaaccccgccgaaagaacccccaggagggactgtataatgagctgcaaaaggacaaaatggcagaagcctattccgaaatagggatgaagggagagcggcggcgaggtaagggacatgacggtctttatcaaggtcttagtactgcaactaaggacacctatgacgcgctgcatatgcaggctctcccacctagataa

SEQ ID NO: 30 - DNA, 1512 bp, synthetic construct
  source 1..1512: mol_type = other DNA
atggccttaccagtgaccgccttgctcctgccgctggccttgctgctccacgccgccaggccgcaagttcagcttgttgaatctggcggcggactggttcagcctggcggatctctgagactgtcttgtgccgccagcggcttcacctttagcagctatgctatgggctgggccagacaggtgccaggcaaagatgtggaatgggtgtccggcatctacagcgacggcagcacctactacgccgactctgtgaagggcagattcaccatcagccggtacaacgccaagaacaccgtgtacctgcagatgaacagcctgaagcctgaggacaccgccgtgtactactgtgccaccgatcctacactggaaaaccagaccacagcctggggccagggaacccaagtgacagtttcttctggcggaggcggatcaggtggcggaggaagcggaggcggcggatctcaagttcaactggttgaaagcggcggaggcctggtccaaccaggtggaagtctgaggctgagctgtaccgcctccggctttagactggattactacgccatcggctggttcagacaggcccctggcaaagagagagaggccatcagctgcatcgacatcaccggcatgcacaccaactacggcgatagcgtgatggggcgcttcaccatctccagagatgacgccaagcggacagtgtatctccagatgaattccctggaagccgaggatacaggcatctactactgcgcccctgctcagtacgccgcctgttctgctctgggcgtgaaggtgtcctttacctcttggggacagggcacacaagtcaccgtgtctccaacaacgacaccagcaccacggccacccactcctgctccgacaattgcgtctcagcccctttcccttcgacccgaagcttgtcgccctgctgcgggaggagcggtccacacgcgcgggcttgacttcgcttgcgacatctacatttgggcacccttggccgggacatgcggcgtcttgctcctgagtctggttataacgctgtattgtaagcgaggtcggaagaagcttttgtatatctttaaacagccctttatgaggcccgtacaaaccacacaagaggaggatgggtgctcatgcagatttcctgaagaggaagagggcggttgcgaacttagagtcaaattcagccgctccgcagatgcacctgcttataaacagggtcagaatcaattgtataatgaacttaatctcgggaggcgcgaggagtatgatgtgctggacaagcgacggggtcgagacccagagatgggcggtaaaccccgccgaaagaacccccaggagggactgtataatgagctgcaaaaggacaaaatggcagaagcctattccgaaatagggatgaagggagagcggcggcgaggtaagggacatgacggtctttatcaaggtcttagtactgcaactaaggacacctatgacgcgctgcatatgcaggctctcccacctagataa

SEQ ID NO: 31 - DNA, 1512 bp, synthetic construct
  source 1..1512: mol_type = other DNA
atggccttaccagtgaccgccttgctcctgccgctggccttgctgctccacgccgccaggccgcaagttcagcttgttgaatctggcggcggactggttcagcctggcggatctctgagactgtcttgtgccgccagcggcttcacctttagcagctatgctatgggctgggccagacaggtgccaggcaaagatgtggaatgggtgtccggcatctacagcgacggcagcacctactacgccgactctgtgaagggcagattcaccatcagccggtacaacgccaagaacaccgtgtacctgcagatgaacagcctgaagcctgaggacaccgccgtgtactactgtgccaccgatcctacactggaaaaccagaccacagcctggggccagggaacccaagtgacagtttcttctggcggaggcggatcaggtggcggaggaagcggaggcggcggatctcaagttcaactggttgaaagcggcggaggcctggtccaaccaggtggaagtctgaggctgagctgtaccgcctccggctttagactggattactacgccatcggctggttcagacaggcccctggcaaagagagagaggccattgcctgcatcgacatcaccggcttccacaccaactacggcgattccgtgtctggccggttcaccatctccagagataatgccggcaccacagtgtatctccagatgaattccctggaagccgaggatacaggcatctactactgcgcccctgccagatacgccgcctgttctgctctggatgtgaagctgtccttcaccagctggggacagggcacacaagtcaccgttagctctacaacgacaccagcaccacggccacccactcctgctccgacaattgcgtctcagcccctttcccttcgacccgaagcttgtcgccctgctgcgggaggagcggtccacacgcgcgggcttgacttcgcttgcgacatctacatttgggcacccttggccgggacatgcggcgtcttgctcctgagtctggttataacgctgtattgtaagcgaggtcggaagaagcttttgtatatctttaaacagccctttatgaggcccgtacaaaccacacaagaggaggatgggtgctcatgcagatttcctgaagaggaagagggcggttgcgaacttagagtcaaattcagccgctccgcagatgcacctgcttataaacagggtcagaatcaattgtataatgaacttaatctcgggaggcgcgaggagtatgatgtgctggacaagcgacggggtcgagacccagagatgggcggtaaaccccgccgaaagaacccccaggagggactgtataatgagctgcaaaaggacaaaatggcagaagcctattccgaaatagggatgaagggagagcggcggcgaggtaagggacatgacggtctttatcaaggtcttagtactgcaactaaggacacctatgacgcgctgcatatgcaggctctcccacctagataa

SEQ ID NO: 32 - DNA, 1512 bp, synthetic construct
  source 1..1512: mol_type = other DNA
atggccttaccagtgaccgccttgctcctgccgctggccttgctgctccacgccgccaggccgcaagttcagcttgttgaatctggcggcggactggttcagcctggcggatctctgagactgagctgtaccgccagcggcttcagactggactactatgccatcggctggttcagacaggcccctggcaaagagagagaggccatcagctgcatcgacatcaccggcatgcacaccaactacggcgatagcgtgatgggcagattcaccatcagccgggacgacgccaagagaaccgtgtacctgcagatgaacagcctggaagccgaggacaccggcatctactattgtgcccctgctcagtacgccgcctgttctgctctgggcgtgaaggtgtcctttacctcttggggccagggcacccaagtgacagtttctccaggtggcggaggatctggcggaggtggaagcggcggaggcggttctcaagtgcaactggttgagtcaggcggaggccttgtgcaacctggtggctcactgagactgtcttgtgccgcctccggcttcacctttagcagctatgctatgggctgggctagacaggtgccaggcaaagaggtggaatgggtgtccggaatctacagcgacggcagcaccaattacgccgactccgtgaaaggccggttcaccatctccagagacaacgccaagaacacagtctatctccagatgaactccctgcggcctgaggatacagccgtgtaccactgtgccaccgatcctaccgtgcacagcgatctgcctgtttggggacagggaaccctggtcacagtgtctagtacaacgacaccagcaccacggccacccactcctgctccgacaattgcgtctcagcccctttcccttcgacccgaagcttgtcgccctgctgcgggaggagcggtccacacgcgcgggcttgacttcgcttgcgacatctacatttgggcacccttggccgggacatgcggcgtcttgctcctgagtctggttataacgctgtattgtaagcgaggtcggaagaagcttttgtatatctttaaacagccctttatgaggcccgtacaaaccacacaagaggaggatgggtgctcatgcagatttcctgaagaggaagagggcggttgcgaacttagagtcaaattcagccgctccgcagatgcacctgcttataaacagggtcagaatcaattgtataatgaacttaatctcgggaggcgcgaggagtatgatgtgctggacaagcgacggggtcgagacccagagatgggcggtaaaccccgccgaaagaacccccaggagggactgtataatgagctgcaaaaggacaaaatggcagaagcctattccgaaatagggatgaagggagagcggcggcgaggtaagggacatgacggtctttatcaaggtcttagtactgcaactaaggacacctatgacgcgctgcatatgcaggctctcccacctagataa

SEQ ID NO: 33 - DNA, 1512 bp, synthetic construct
  source 1..1512: mol_type = other DNA
atggccttaccagtgaccgccttgctcctgccgctggccttgctgctccacgccgccaggccgcaagttcagcttgttgaatctggcggcggactggttcagcctggcggatctctgagactgagctgtaccgccagcggcttcagactggactactatgccatcggctggttcagacaggcccctggcaaagagagagaggccatcagctgcatcgacatcaccggcatgcacaccaactacggcgatagcgtgatgggcagattcaccatcagccgggacgacgccaagagaaccgtgtacctgcagatgaacagcctggaagccgaggacaccggcatctactattgtgcccctgctcagtacgccgcctgttctgctctgggcgtgaaggtgtcctttacctcttggggccagggcacccaagtgacagtttctccaggtggcggaggatctggcggaggtggaagcggcggaggcggttctcaagtgcaactggttgagtcaggcggaggccttgtgcaacctggtggctcactgagactgtcttgtgccgcctccggcttcacctttagcagctatgctatgggctgggctagacaggtgcccggcaaagatgtggaatgggtgtccggaatctacagcgacggcagcacctactacgccgactctgtgaaaggccggttcaccatctccagatacaacgccaagaacacagtctacctccaaatgaactccctcaagcctgaggataccgccgtgtactactgcgccaccgatcctacactggaaaaccagaccacagcctggggacagggaacacaagtcaccgtgtcaagcacaacgacaccagcaccacggccacccactcctgctccgacaattgcgtctcagcccctttcccttcgacccgaagcttgtcgccctgctgcgggaggagcggtccacacgcgcgggcttgacttcgcttgcgacatctacatttgggcacccttggccgggacatgcggcgtcttgctcctgagtctggttataacgctgtattgtaagcgaggtcggaagaagcttttgtatatctttaaacagccctttatgaggcccgtacaaaccacacaagaggaggatgggtgctcatgcagatttcctgaagaggaagagggcggttgcgaacttagagtcaaattcagccgctccgcagatgcacctgcttataaacagggtcagaatcaattgtataatgaacttaatctcgggaggcgcgaggagtatgatgtgctggacaagcgacggggtcgagacccagagatgggcggtaaaccccgccgaaagaacccccaggagggactgtataatgagctgcaaaaggacaaaatggcagaagcctattccgaaatagggatgaagggagagcggcggcgaggtaagggacatgacggtctttatcaaggtcttagtactgcaactaaggacacctatgacgcgctgcatatgcaggctctcccacctagataa

SEQ ID NO: 34 - DNA, 1512 bp, synthetic construct
  source 1..1512: mol_type = other DNA
atggccttaccagtgaccgccttgctcctgccgctggccttgctgctccacgccgccaggccgcaagttcagcttgttgaatctggcggcggactggttcagcctggcggatctctgagactgagctgtaccgccagcggcttcagactggactactatgccatcggctggttcagacaggcccctggcaaagagagagaggccattgcctgcatcgacatcaccggcttccacaccaactacggcgatagcgtgtccggcagattcaccatcagcagagacaatgccggcaccaccgtgtacctgcagatgaactctctggaagccgaggacaccggcatctactactgtgcccctgccagatacgccgcctgttctgccctggatgtgaagctgagctttacctcttggggccagggcacccaagtgacagtttcttctggtggcggaggatctggcggaggtggaagcggcggaggcggttctcaagtgcaactggttgagtcaggcggaggccttgtgcaacctggtggctcactgagactgtcttgtgccgcctccggcttcacctttagcagctatgctatgggctgggctagacaggtgccaggcaaagaggtggaatgggtgtccggaatctacagcgacggcagcaccaattacgccgactccgtgaagggacgcttcacaatctcccgggacaacgccaagaacacagtgtatctccaaatgaacagcctgcggcctgaggataccgccgtgtaccattgtgccaccgatcctaccgtgcacagcgatctgcctgtttggggacagggaaccctggtcacagtgtctagtacaacgacaccagcaccacggccacccactcctgctccgacaattgcgtctcagcccctttcccttcgacccgaagcttgtcgccctgctgcgggaggagcggtccacacgcgcgggcttgacttcgcttgcgacatctacatttgggcacccttggccgggacatgcggcgtcttgctcctgagtctggttataacgctgtattgtaagcgaggtcggaagaagcttttgtatatctttaaacagccctttatgaggcccgtacaaaccacacaagaggaggatgggtgctcatgcagatttcctgaagaggaagagggcggttgcgaacttagagtcaaattcagccgctccgcagatgcacctgcttataaacagggtcagaatcaattgtataatgaacttaatctcgggaggcgcgaggagtatgatgtgctggacaagcgacggggtcgagacccagagatgggcggtaaaccccgccgaaagaacccccaggagggactgtataatgagctgcaaaaggacaaaatggcagaagcctattccgaaatagggatgaagggagagcggcggcgaggtaagggacatgacggtctttatcaaggtcttagtactgcaactaaggacacctatgacgcgctgcatatgcaggctctcccacctagataa

SEQ ID NO: 35 - DNA, 1512 bp, synthetic construct
  source 1..1512: mol_type = other DNA
atggccttaccagtgaccgccttgctcctgccgctggccttgctgctccacgccgccaggccgcaagttcagcttgttgaatctggcggcggactggttcagcctggcggatctctgagactgagctgtaccgccagcggcttcagactggactactatgccatcggctggttcagacaggcccctggcaaagagagagaggccattgcctgcatcgacatcaccggcttccacaccaactacggcgatagcgtgtccggcagattcaccatcagcagagacaatgccggcaccaccgtgtacctgcagatgaactctctggaagccgaggacaccggcatctactactgtgcccctgccagatacgccgcctgttctgccctggatgtgaagctgagctttacctcttggggccagggcacccaagtgacagtttcttctggtggcggaggatctggcggaggtggaagcggcggaggcggttctcaagtgcaactggttgagtcaggcggaggccttgtgcaacctggtggctcactgagactgtcttgtgccgcctccggcttcacctttagcagctatgctatgggctgggctagacaggtgcccggcaaagatgtggaatgggtgtccggaatctacagcgacggcagcacctactacgccgactctgtgaagggacgcttcaccatctccagatacaacgccaagaacacagtctacctccaaatgaacagcctgaagcctgaggataccgccgtgtactattgcgccaccgatcctacactggaaaaccagacaacagcctggggacagggaacacaagtcaccgtgtcaagcacaacgacaccagcaccacggccacccactcctgctccgacaattgcgtctcagcccctttcccttcgacccgaagcttgtcgccctgctgcgggaggagcggtccacacgcgcgggcttgacttcgcttgcgacatctacatttgggcacccttggccgggacatgcggcgtcttgctcctgagtctggttataacgctgtattgtaagcgaggtcggaagaagcttttgtatatctttaaacagccctttatgaggcccgtacaaaccacacaagaggaggatgggtgctcatgcagatttcctgaagaggaagagggcggttgcgaacttagagtcaaattcagccgctccgcagatgcacctgcttataaacagggtcagaatcaattgtataatgaacttaatctcgggaggcgcgaggagtatgatgtgctggacaagcgacggggtcgagacccagagatgggcggtaaaccccgccgaaagaacccccaggagggactgtataatgagctgcaaaaggacaaaatggcagaagcctattccgaaatagggatgaagggagagcggcggcgaggtaagggacatgacggtctttatcaaggtcttagtactgcaactaaggacacctatgacgcgctgcatatgcaggctctcccacctagataa

SEQ ID NO: 36 - DNA, 1482 bp, synthetic construct
  source 1..1482: mol_type = other DNA
atggccttaccagtgaccgccttgctcctgccgctggccttgctgctccacgccgccaggccgcaagttcagcttgttgaatctggcggcggactggttcagcctggcggatctctgagactgtcttgtgccgccagcggcttcacctttagcagctatgctatgggctgggccagacaggtgccaggcaaagaggttgaatgggtgtccggcatctacagcgacggcagcaccaattacgccgacagcgtgaagggcagattcaccatcagccgggacaacgccaagaacaccgtgtacctgcagatgaacagcctgcggcctgaggatacagccgtgtaccactgtgccaccgatcctaccgtgcacagcgatctgcctgtttggggacagggcacactggtcacagtttctagcggaggcggaggatcaggtggcggtggatctggcggtggtggttctcaagtgcagctcgtggaaagcggcggcgggctcgtgcaagccggggggagcctgagactggcctgcaccgctagcggcaacatcttcgctagccaagtgatgaactggtacagacaagcccccggcagccctagagagctggtggccaccatcacccccggcggcagaaccacctacgccgacagcgccaagggcagattcaccgtggccaccgacaacgccaaggccaccgcctacctgcagctgacaagcctgacccccgaggataccggcgtgtactactgccacgtgagactgttccccgccaccgactactggggccaaggcacccaagtgaccgtgagcagcacaacgacaccagcaccacggccacccactcctgctccgacaattgcgtctcagcccctttcccttcgacccgaagcttgtcgccctgctgcgggaggagcggtccacacgcgcgggcttgacttcgcttgcgacatctacatttgggcacccttggccgggacatgcggcgtcttgctcctgagtctggttataacgctgtattgtaagcgaggtcggaagaagcttttgtatatctttaaacagccctttatgaggcccgtacaaaccacacaagaggaggatgggtgctcatgcagatttcctgaagaggaagagggcggttgcgaacttagagtcaaattcagccgctccgcagatgcacctgcttataaacagggtcagaatcaattgtataatgaacttaatctcgggaggcgcgaggagtatgatgtgctggacaagcgacggggtcgagacccagagatgggcggtaaaccccgccgaaagaacccccaggagggactgtataatgagctgcaaaaggacaaaatggcagaagcctattccgaaatagggatgaagggagagcggcggcgaggtaagggacatgacggtctttatcaaggtcttagtactgcaactaaggacacctatgacgcgctgcatatgcaggctctcccacctagataa

SEQ ID NO: 37 - DNA, 1482 bp, synthetic construct
  source 1..1482: mol_type = other DNA
atggccttaccagtgaccgccttgctcctgccgctggccttgctgctccacgccgccaggccgcaagttcagcttgttgaatctggcggcggactggttcagcctggcggatctctgagactgtcttgtgccgccagcggcttcacctttagcagctatgctatgggctgggccagacaggtgccaggcaaagatgtggaatgggtgtccggcatctacagcgacggcagcacctactacgccgactctgtgaagggcagattcaccatcagccggtacaacgccaagaacaccgtgtacctgcagatgaacagcctgaagcctgaggacaccgccgtgtactactgtgccaccgatcctacactggaaaaccagaccacagcctggggccagggaacccaagtgacagtttcttctggcggaggcggatcaggtggcggaggaagcggaggcggcggatctcaagtgcagctcgtggaaagcggcggcgggctcgtgcaagccggggggagcctgagactggcctgcaccgctagcggcaacatcttcgctagccaagtgatgaactggtacagacaagcccccggcagccctagagagctggtggccaccatcacccccggcggcagaaccacctacgccgacagcgccaagggcagattcaccgtggccaccgacaacgccaaggccaccgcctacctgcagctgacaagcctgacccccgaggataccggcgtgtactactgccacgtgagactgttccccgccaccgactactggggccaaggcacccaagtgaccgtgagcagcacaacgacaccagcaccacggccacccactcctgctccgacaattgcgtctcagcccctttcccttcgacccgaagcttgtcgccctgctgcgggaggagcggtccacacgcgcgggcttgacttcgcttgcgacatctacatttgggcacccttggccgggacatgcggcgtcttgctcctgagtctggttataacgctgtattgtaagcgaggtcggaagaagcttttgtatatctttaaacagccctttatgaggcccgtacaaaccacacaagaggaggatgggtgctcatgcagatttcctgaagaggaagagggcggttgcgaacttagagtcaaattcagccgctccgcagatgcacctgcttataaacagggtcagaatcaattgtataatgaacttaatctcgggaggcgcgaggagtatgatgtgctggacaagcgacggggtcgagacccagagatgggcggtaaaccccgccgaaagaacccccaggagggactgtataatgagctgcaaaaggacaaaatggcagaagcctattccgaaatagggatgaagggagagcggcggcgaggtaagggacatgacggtctttatcaaggtcttagtactgcaactaaggacacctatgacgcgctgcatatgcaggctctcccacctagataa

SEQ ID NO: 38 - DNA, 1482 bp, synthetic construct
  source 1..1482: mol_type = other DNA
atggccttaccagtgaccgccttgctcctgccgctggccttgctgctccacgccgccaggccgcaagtgcagctcgtggaaagcggcggcgggctcgtgcaagccggggggagcctgagactggcctgcaccgctagcggcaacatcttcgctagccaagtgatgaactggtacagacaagcccccggcagccctagagagctggtggccaccatcacccccggcggcagaaccacctacgccgacagcgccaagggcagattcaccgtggccaccgacaacgccaaggccaccgcctacctgcagctgacaagcctgacccccgaggataccggcgtgtactactgccacgtgagactgttccccgccaccgactactggggccaaggcacccaagtgaccgtgagcagcggtggcggaggatctggcggaggtggaagcggcggaggcggttctcaagtgcaactggttgagtcaggcggaggccttgtgcaacctggtggctcactgagactgtcttgtgccgcctccggcttcacctttagcagctatgctatgggctgggctagacaggtgccaggcaaagaggtggaatgggtgtccggaatctacagcgacggcagcaccaattacgccgactccgtgaaaggccggttcaccatctccagagacaacgccaagaacacagtctatctccagatgaactccctgcggcctgaggatacagccgtgtaccactgtgccaccgatcctaccgtgcacagcgatctgcctgtttggggacagggaaccctggtcacagtgtctagtacaacgacaccagcaccacggccacccactcctgctccgacaattgcgtctcagcccctttcccttcgacccgaagcttgtcgccctgctgcgggaggagcggtccacacgcgcgggcttgacttcgcttgcgacatctacatttgggcacccttggccgggacatgcggcgtcttgctcctgagtctggttataacgctgtattgtaagcgaggtcggaagaagcttttgtatatctttaaacagccctttatgaggcccgtacaaaccacacaagaggaggatgggtgctcatgcagatttcctgaagaggaagagggcggttgcgaacttagagtcaaattcagccgctccgcagatgcacctgcttataaacagggtcagaatcaattgtataatgaacttaatctcgggaggcgcgaggagtatgatgtgctggacaagcgacggggtcgagacccagagatgggcggtaaaccccgccgaaagaacccccaggagggactgtataatgagctgcaaaaggacaaaatggcagaagcctattccgaaatagggatgaagggagagcggcggcgaggtaagggacatgacggtctttatcaaggtcttagtactgcaactaaggacacctatgacgcgctgcatatgcaggctctcccacctagataa

SEQ ID NO: 39 - DNA, 1482 bp, synthetic construct
  source 1..1482: mol_type = other DNA
atggccttaccagtgaccgccttgctcctgccgctggccttgctgctccacgccgccaggccgcaagtgcagctcgtggaaagcggcggcgggctcgtgcaagccggggggagcctgagactggcctgcaccgctagcggcaacatcttcgctagccaagtgatgaactggtacagacaagcccccggcagccctagagagctggtggccaccatcacccccggcggcagaaccacctacgccgacagcgccaagggcagattcaccgtggccaccgacaacgccaaggccaccgcctacctgcagctgacaagcctgacccccgaggataccggcgtgtactactgccacgtgagactgttccccgccaccgactactggggccaaggcacccaagtgaccgtgagcagcggtggcggaggatctggcggaggtggaagcggcggaggcggttctcaagtgcaactggttgagtcaggcggaggccttgtgcaacctggtggctcactgagactgtcttgtgccgcctccggcttcacctttagcagctatgctatgggctgggctagacaggtgcccggcaaagatgtggaatgggtgtccggaatctacagcgacggcagcacctactacgccgactctgtgaaaggccggttcaccatctccagatacaacgccaagaacacagtctacctccaaatgaactccctcaagcctgaggataccgccgtgtactactgcgccaccgatcctacactggaaaaccagaccacagcctggggacagggaacacaagtcaccgtgtcaagcacaacgacaccagcaccacggccacccactcctgctccgacaattgcgtctcagcccctttcccttcgacccgaagcttgtcgccctgctgcgggaggagcggtccacacgcgcgggcttgacttcgcttgcgacatctacatttgggcacccttggccgggacatgcggcgtcttgctcctgagtctggttataacgctgtattgtaagcgaggtcggaagaagcttttgtatatctttaaacagccctttatgaggcccgtacaaaccacacaagaggaggatgggtgctcatgcagatttcctgaagaggaagagggcggttgcgaacttagagtcaaattcagccgctccgcagatgcacctgcttataaacagggtcagaatcaattgtataatgaacttaatctcgggaggcgcgaggagtatgatgtgctggacaagcgacggggtcgagacccagagatgggcggtaaaccccgccgaaagaacccccaggagggactgtataatgagctgcaaaaggacaaaatggcagaagcctattccgaaatagggatgaagggagagcggcggcgaggtaagggacatgacggtctttatcaaggtcttagtactgcaactaaggacacctatgacgcgctgcatatgcaggctctcccacctagataa

SEQ ID NO: 40 - DNA, 2034 bp, synthetic construct
  source 1..2034: mol_type = other DNA
atggctctgcctgtgacagctctgctgctgcctctggctctgcttctgcatgccgccagaccgcaagtgcaactcgtggagagcgggggggggctggtgcagcccggggggagcctgagactgagctgcgccgctagcggcttcaccttcagcagctacgccatgggctgggctagacaagtgcccggcaaagaggtggagtgggtgagcggcatctacagcgacggcagcaccaactacgccgacagcgtgaagggcagattcaccatcagcagagacaacgccaagaacaccgtgtacctgcagatgaacagcctgagacccgaggacaccgccgtgtaccactgcgccacagatcccacagtgcacagcgatctgcccgtctgggggcaaggcaccctggtcaccgtgagcagcggaagcactagcggaagcggaaagccaggaagcggagaaggaagcactaagggacaagtgcagctcgtggaaagcggcggcgggctcgtgcaagccggggggagcctgagactggcctgcaccgctagcggcaacatcttcgctagccaagtgatgaactggtacagacaagcccccggcagccctagagagctggtggccaccatcacccccggcggcagaaccacctacgccgacagcgccaagggcagattcaccgtggccaccgacaacgccaaggccaccgcctacctgcagctgacaagcctgctggaggccgaggacaccggcatctactactgcgcccccgctagatacgccgcctgcagcgccctggacgtgaagctgagcttcacaagctggggccaaggcacccaagtgaccgtgagcagcgccgaggatctggccgtgtactactgccagaacgactacagctaccccttcacctttggcagcggcaccaagctggaaatcaaaggcggaggcggatctggcggcggaggtagcggtggcggaggatctcaagttcagctgcaacagcctggcgccgaactcgttagacctggcgcttctgtgaagctgtcctgcaaggccagcggctacacctttaccagctactggatcaactgggtcaagcagaggccaggccagggcctcgaatggatcggcaatatctaccccagcgacagctacaccaactacaatcagaagttcaaggacaaggccacactgaccgtggacaagtctagcagcaccgcctacatgcagctgagcagccctacaagcgaggacagcgccgtgtattattgcacccggtcttggcggggcaacagcttcgattattggggccagggcacaaccctgaccgtgtctagcaccaccaccgactacaaggacgacgacgacaagcccgctcctagacctcctacaccagctcctacaatcgccagccagcctctgtctctgaggccagaagcttgtagacctgctgctggcggagccgtgcatacaagaggactggatttcgcctgcgacttctgggtgctcgtggttgttggcggagtgctggcctgttactctctgctggtcaccgtggccttcatcatcttttgggtccgaagcaagcggagccggctgctgcacagcgactacatgaacatgacccctagacggcccggacctaccagaaagcactaccagccttacgctcctcctagagacttcgccgcctaccggtccagagtgaagttcagcagatccgctgatgcccctgcctatcagcagggccagaaccagctgtacaacgagctgaacctggggagaagagaagagtacgacgtgctggacaagcggagaggcagagatcctgagatgggcggcaagcccagacggaagaatcctcaagagggcctgtacaatgaactgcagaaagacaagatggccgaggcctacagcgagatcggaatgaagggcgagcgcagaagaggcaagggacacgatggactgtaccagggcctgagcaccgccaccaaggatacctatgatgccctgcacatgcaggccctgcctccaagataa

SEQ ID NO: 41 - DNA, 2034 bp, synthetic construct
  source 1..2034: mol_type = other DNA
atggctctgcctgtgacagctctgctgctgcctctggctctgcttctgcatgccgccagaccgcaagtgcaactcgtggagagcgggggggggctggtgcagcccggggggagcctgagactgagctgcgccgctagcggcttcaccttcagcagctacgccatgggctgggctagacaagtgcccggcaaagaggtggagtgggtgagcggcatctacagcgacggcagcaccaactacgccgacagcgtgaagggcagattcaccatcagcagagacaacgccaagaacaccgtgtacctgcagatgaacagcctgagacccgaggacaccgccgtgtaccactgcgccacagatcccacagtgcacagcgatctgcccgtctgggggcaaggcaccctggtcaccgtgagcagcggaagcactagcggaagcggaaagccaggaagcggagaaggaagcactaagggacaagtgcaactcgtcgaaagcggcggcgggctcgtgcaacctggggggagcctgagactgagctgcaccgctagcggcttcagactggactactacgccatcggctggttcagacaagcccccggcaaggagagagaggccatcagctgcatcgacatcaccggcatgcacaccaactacggcgacagcgtgatgggcagattcaccatcagcagagacgacgccaagagaaccgtgtacctgcagatgaacagcctggaggccgaggacaccggcatctactactgcgcccccgctcagtacgccgcctgcagcgccctgggcgtgaaggtgagcttcacaagctggggccaaggcacccaagtgaccgtgagccccgccgaggatctggccgtgtactactgccagaacgactacagctaccccttcacctttggcagcggcaccaagctggaaatcaaaggcggaggcggatctggcggcggaggtagcggtggcggaggatctcaagttcagctgcaacagcctggcgccgaactcgttagacctggcgcttctgtgaagctgtcctgcaaggccagcggctacacctttaccagctactggatcaactgggtcaagcagaggccaggccagggcctcgaatggatcggcaatatctaccccagcgacagctacaccaactacaatcagaagttcaaggacaaggccacactgaccgtggacaagtctagcagcaccgcctacatgcagctgagcagccctacaagcgaggacagcgccgtgtattattgcacccggtcttggcggggcaacagcttcgattattggggccagggcacaaccctgaccgtgtctagcaccaccaccgactacaaggacgacgacgacaagcccgctcctagacctcctacaccagctcctacaatcgccagccagcctctgtctctgaggccagaagcttgtagacctgctgctggcggagccgtgcatacaagaggactggatttcgcctgcgacttctgggtgctcgtggttgttggcggagtgctggcctgttactctctgctggtcaccgtggccttcatcatcttttgggtccgaagcaagcggagccggctgctgcacagcgactacatgaacatgacccctagacggcccggacctaccagaaagcactaccagccttacgctcctcctagagacttcgccgcctaccggtccagagtgaagttcagcagatccgctgatgcccctgcctatcagcagggccagaaccagctgtacaacgagctgaacctggggagaagagaagagtacgacgtgctggacaagcggagaggcagagatcctgagatgggcggcaagcccagacggaagaatcctcaagagggcctgtacaatgaactgcagaaagacaagatggccgaggcctacagcgagatcggaatgaagggcgagcgcagaagaggcaagggacacgatggactgtaccagggcctgagcaccgccaccaaggatacctatgatgccctgcacatgcaggccctgcctccaagataa

SEQ ID NO: 42 - DNA, 2034 bp, synthetic construct
  source 1..2034: mol_type = other DNA
atggctctgcctgtgacagctctgctgctgcctctggctctgcttctgcatgccgccagaccgcaagtgcaactcgtggagagcgggggggggctggtgcagcccggggggagcctgagactgagctgcgccgctagcggcttcaccttcagcagctacgccatgggctgggctagacaagtgcccggcaaagaggtggagtgggtgagcggcatctacagcgacggcagcaccaactacgccgacagcgtgaagggcagattcaccatcagcagagacaacgccaagaacaccgtgtacctgcagatgaacagcctgagacccgaggacaccgccgtgtaccactgcgccacagatcccacagtgcacagcgatctgcccgtctgggggcaaggcaccctggtcaccgtgagcagcggaagcactagcggaagcggaaagccaggaagcggagaaggaagcactaagggacaagtgcaactcgtcgaaagcggcggcgggctcgtgcaacctggggggagcctgagactgagctgcaccgctagcggcttcagactggactactacgccatcggctggttcagacaagcccccggcaaggagagagaggccatcgcctgcatcgacatcaccggcttccacaccaactacggcgacagcgtgagcggcagattcaccatcagcagagacaacgccggcaccaccgtgtacctgcagatgaacagcctggaggccgaggacaccggcatctactactgcgcccccgctagatacgccgcctgcagcgccctggacgtgaagctgagcttcacaagctggggccaaggcacccaagtgaccgtgagcagcgccgaggatctggccgtgtactactgccagaacgactacagctaccccttcacctttggcagcggcaccaagctggaaatcaaaggcggaggcggatctggcggcggaggtagcggtggcggaggatctcaagttcagctgcaacagcctggcgccgaactcgttagacctggcgcttctgtgaagctgtcctgcaaggccagcggctacacctttaccagctactggatcaactgggtcaagcagaggccaggccagggcctcgaatggatcggcaatatctaccccagcgacagctacaccaactacaatcagaagttcaaggacaaggccacactgaccgtggacaagtctagcagcaccgcctacatgcagctgagcagccctacaagcgaggacagcgccgtgtattattgcacccggtcttggcggggcaacagcttcgattattggggccagggcacaaccctgaccgtgtctagcaccaccaccgactacaaggacgacgacgacaagcccgctcctagacctcctacaccagctcctacaatcgccagccagcctctgtctctgaggccagaagcttgtagacctgctgctggcggagccgtgcatacaagaggactggatttcgcctgcgacttctgggtgctcgtggttgttggcggagtgctggcctgttactctctgctggtcaccgtggccttcatcatcttttgggtccgaagcaagcggagccggctgctgcacagcgactacatgaacatgacccctagacggcccggacctaccagaaagcactaccagccttacgctcctcctagagacttcgccgcctaccggtccagagtgaagttcagcagatccgctgatgcccctgcctatcagcagggccagaaccagctgtacaacgagctgaacctggggagaagagaagagtacgacgtgctggacaagcggagaggcagagatcctgagatgggcggcaagcccagacggaagaatcctcaagagggcctgtacaatgaactgcagaaagacaagatggccgaggcctacagcgagatcggaatgaagggcgagcgcagaagaggcaagggacacgatggactgtaccagggcctgagcaccgccaccaaggatacctatgatgccctgcacatgcaggccctgcctccaagataa

SEQ ID NO: 43 - DNA, 2034 bp, synthetic construct
  source 1..2034: mol_type = other DNA
atggctctgcctgtgacagctctgctgctgcctctggctctgcttctgcatgccgccagaccgcaagtgcagctggtcgagagcggcgggggcctcgtccaacccggcggcagcctgagactgagctgcgccgctagcggcttcaccttcagcagctacgccatgggctgggctagacaagtgcccggcaaggacgtggagtgggtgagcggcatctacagcgacggcagcacctactacgccgacagcgtgaagggcagattcaccatcagcagatacaacgccaagaacaccgtgtacctgcagatgaacagcctgaagcccgaggacaccgccgtgtactactgcgccaccgatcctaccctcgagaatcagacaaccgcctggggccaagggacccaagtgaccgtgagcagcggaagcactagcggaagcggaaagccaggaagcggagaaggaagcactaagggacaagtgcagctcgtggaaagcggcggcgggctcgtgcaagccggggggagcctgagactggcctgcaccgctagcggcaacatcttcgctagccaagtgatgaactggtacagacaagcccccggcagccctagagagctggtggccaccatcacccccggcggcagaaccacctacgccgacagcgccaagggcagattcaccgtggccaccgacaacgccaaggccaccgcctacctgcagctgacaagcctgctggaggccgaggacaccggcatctactactgcgcccccgctagatacgccgcctgcagcgccctggacgtgaagctgagcttcacaagctggggccaaggcacccaagtgaccgtgagcagcgccgaggatctggccgtgtactactgccagaacgactacagctaccccttcacctttggcagcggcaccaagctggaaatcaaaggcggaggcggatctggcggcggaggtagcggtggcggaggatctcaagttcagctgcaacagcctggcgccgaactcgttagacctggcgcttctgtgaagctgtcctgcaaggccagcggctacacctttaccagctactggatcaactgggtcaagcagaggccaggccagggcctcgaatggatcggcaatatctaccccagcgacagctacaccaactacaatcagaagttcaaggacaaggccacactgaccgtggacaagtctagcagcaccgcctacatgcagctgagcagccctacaagcgaggacagcgccgtgtattattgcacccggtcttggcggggcaacagcttcgattattggggccagggcacaaccctgaccgtgtctagcaccaccaccgactacaaggacgacgacgacaagcccgctcctagacctcctacaccagctcctacaatcgccagccagcctctgtctctgaggccagaagcttgtagacctgctgctggcggagccgtgcatacaagaggactggatttcgcctgcgacttctgggtgctcgtggttgttggcggagtgctggcctgttactctctgctggtcaccgtggccttcatcatcttttgggtccgaagcaagcggagccggctgctgcacagcgactacatgaacatgacccctagacggcccggacctaccagaaagcactaccagccttacgctcctcctagagacttcgccgcctaccggtccagagtgaagttcagcagatccgctgatgcccctgcctatcagcagggccagaaccagctgtacaacgagctgaacctggggagaagagaagagtacgacgtgctggacaagcggagaggcagagatcctgagatgggcggcaagcccagacggaagaatcctcaagagggcctgtacaatgaactgcagaaagacaagatggccgaggcctacagcgagatcggaatgaagggcgagcgcagaagaggcaagggacacgatggactgtaccagggcctgagcaccgccaccaaggatacctatgatgccctgcacatgcaggccctgcctccaagataa

SEQ ID NO: 44 - DNA, 2034 bp, synthetic construct
  source 1..2034: mol_type = other DNA
atggctctgcctgtgacagctctgctgctgcctctggctctgcttctgcatgccgccagaccgcaagtgcagctggtcgagagcggcgggggcctcgtccaacccggcggcagcctgagactgagctgcgccgctagcggcttcaccttcagcagctacgccatgggctgggctagacaagtgcccggcaaggacgtggagtgggtgagcggcatctacagcgacggcagcacctactacgccgacagcgtgaagggcagattcaccatcagcagatacaacgccaagaacaccgtgtacctgcagatgaacagcctgaagcccgaggacaccgccgtgtactactgcgccaccgatcctaccctcgagaatcagacaaccgcctggggccaagggacccaagtgaccgtgagcagcggaagcactagcggaagcggaaagccaggaagcggagaaggaagcactaagggacaagtgcaactcgtcgaaagcggcggcgggctcgtgcaacctggggggagcctgagactgagctgcaccgctagcggcttcagactggactactacgccatcggctggttcagacaagcccccggcaaggagagagaggccatcagctgcatcgacatcaccggcatgcacaccaactacggcgacagcgtgatgggcagattcaccatcagcagagacgacgccaagagaaccgtgtacctgcagatgaacagcctggaggccgaggacaccggcatctactactgcgcccccgctcagtacgccgcctgcagcgccctgggcgtgaaggtgagcttcacaagctggggccaaggcacccaagtgaccgtgagccccgccgaggatctggccgtgtactactgccagaacgactacagctaccccttcacctttggcagcggcaccaagctggaaatcaaaggcggaggcggatctggcggcggaggtagcggtggcggaggatctcaagttcagctgcaacagcctggcgccgaactcgttagacctggcgcttctgtgaagctgtcctgcaaggccagcggctacacctttaccagctactggatcaactgggtcaagcagaggccaggccagggcctcgaatggatcggcaatatctaccccagcgacagctacaccaactacaatcagaagttcaaggacaaggccacactgaccgtggacaagtctagcagcaccgcctacatgcagctgagcagccctacaagcgaggacagcgccgtgtattattgcacccggtcttggcggggcaacagcttcgattattggggccagggcacaaccctgaccgtgtctagcaccaccaccgactacaaggacgacgacgacaagcccgctcctagacctcctacaccagctcctacaatcgccagccagcctctgtctctgaggccagaagcttgtagacctgctgctggcggagccgtgcatacaagaggactggatttcgcctgcgacttctgggtgctcgtggttgttggcggagtgctggcctgttactctctgctggtcaccgtggccttcatcatcttttgggtccgaagcaagcggagccggctgctgcacagcgactacatgaacatgacccctagacggcccggacctaccagaaagcactaccagccttacgctcctcctagagacttcgccgcctaccggtccagagtgaagttcagcagatccgctgatgcccctgcctatcagcagggccagaaccagctgtacaacgagctgaacctggggagaagagaagagtacgacgtgctggacaagcggagaggcagagatcctgagatgggcggcaagcccagacggaagaatcctcaagagggcctgtacaatgaactgcagaaagacaagatggccgaggcctacagcgagatcggaatgaagggcgagcgcagaagaggcaagggacacgatggactgtaccagggcctgagcaccgccaccaaggatacctatgatgccctgcacatgcaggccctgcctccaagataa

SEQ ID NO: 45 - DNA, 2034 bp, synthetic construct
  source 1..2034: mol_type = other DNA
atggctctgcctgtgacagctctgctgctgcctctggctctgcttctgcatgccgccagaccgcaagtgcagctggtcgagagcggcgggggcctcgtccaacccggcggcagcctgagactgagctgcgccgctagcggcttcaccttcagcagctacgccatgggctgggctagacaagtgcccggcaaggacgtggagtgggtgagcggcatctacagcgacggcagcacctactacgccgacagcgtgaagggcagattcaccatcagcagatacaacgccaagaacaccgtgtacctgcagatgaacagcctgaagcccgaggacaccgccgtgtactactgcgccaccgatcctaccctcgagaatcagacaaccgcctggggccaagggacccaagtgaccgtgagcagcggaagcactagcggaagcggaaagccaggaagcggagaaggaagcactaagggacaagtgcaactcgtcgaaagcggcggcgggctcgtgcaacctggggggagcctgagactgagctgcaccgctagcggcttcagactggactactacgccatcggctggttcagacaagcccccggcaaggagagagaggccatcgcctgcatcgacatcaccggcttccacaccaactacggcgacagcgtgagcggcagattcaccatcagcagagacaacgccggcaccaccgtgtacctgcagatgaacagcctggaggccgaggacaccggcatctactactgcgcccccgctagatacgccgcctgcagcgccctggacgtgaagctgagcttcacaagctggggccaaggcacccaagtgaccgtgagcagcgccgaggatctggccgtgtactactgccagaacgactacagctaccccttcacctttggcagcggcaccaagctggaaatcaaaggcggaggcggatctggcggcggaggtagcggtggcggaggatctcaagttcagctgcaacagcctggcgccgaactcgttagacctggcgcttctgtgaagctgtcctgcaaggccagcggctacacctttaccagctactggatcaactgggtcaagcagaggccaggccagggcctcgaatggatcggcaatatctaccccagcgacagctacaccaactacaatcagaagttcaaggacaaggccacactgaccgtggacaagtctagcagcaccgcctacatgcagctgagcagccctacaagcgaggacagcgccgtgtattattgcacccggtcttggcggggcaacagcttcgattattggggccagggcacaaccctgaccgtgtctagcaccaccaccgactacaaggacgacgacgacaagcccgctcctagacctcctacaccagctcctacaatcgccagccagcctctgtctctgaggccagaagcttgtagacctgctgctggcggagccgtgcatacaagaggactggatttcgcctgcgacttctgggtgctcgtggttgttggcggagtgctggcctgttactctctgctggtcaccgtggccttcatcatcttttgggtccgaagcaagcggagccggctgctgcacagcgactacatgaacatgacccctagacggcccggacctaccagaaagcactaccagccttacgctcctcctagagacttcgccgcctaccggtccagagtgaagttcagcagatccgctgatgcccctgcctatcagcagggccagaaccagctgtacaacgagctgaacctggggagaagagaagagtacgacgtgctggacaagcggagaggcagagatcctgagatgggcggcaagcccagacggaagaatcctcaagagggcctgtacaatgaactgcagaaagacaagatggccgaggcctacagcgagatcggaatgaagggcgagcgcagaagaggcaagggacacgatggactgtaccagggcctgagcaccgccaccaaggatacctatgatgccctgcacatgcaggccctgcctccaagataa

SEQ ID NO: 46 - DNA, 2034 bp, synthetic construct
  source 1..2034: mol_type = other DNA
atggctctgcctgtgacagctctgctgctgcctctggctctgcttctgcatgccgccagaccgcaagtgcagctcgtggaaagcggcggcgggctcgtgcaagccggggggagcctgagactggcctgcaccgctagcggcaacatcttcgctagccaagtgatgaactggtacagacaagcccccggcagccctagagagctggtggccaccatcacccccggcggcagaaccacctacgccgacagcgccaagggcagattcaccgtggccaccgacaacgccaaggccaccgcctacctgcagctgacaagcctgctggaggccgaggacaccggcatctactactgcgcccccgctagatacgccgcctgcagcgccctggacgtgaagctgagcttcacaagctggggccaaggcacccaagtgaccgtgagcagcggaagcactagcggaagcggaaagccaggaagcggagaaggaagcactaagggacaagtgcaactcgtggagagcgggggggggctggtgcagcccggggggagcctgagactgagctgcgccgctagcggcttcaccttcagcagctacgccatgggctgggctagacaagtgcccggcaaagaggtggagtgggtgagcggcatctacagcgacggcagcaccaactacgccgacagcgtgaagggcagattcaccatcagcagagacaacgccaagaacaccgtgtacctgcagatgaacagcctgagacccgaggacaccgccgtgtaccactgcgccacagatcccacagtgcacagcgatctgcccgtctgggggcaaggcaccctggtcaccgtgagcagcgccgaggatctggccgtgtactactgccagaacgactacagctaccccttcacctttggcagcggcaccaagctggaaatcaaaggcggaggcggatctggcggcggaggtagcggtggcggaggatctcaagttcagctgcaacagcctggcgccgaactcgttagacctggcgcttctgtgaagctgtcctgcaaggccagcggctacacctttaccagctactggatcaactgggtcaagcagaggccaggccagggcctcgaatggatcggcaatatctaccccagcgacagctacaccaactacaatcagaagttcaaggacaaggccacactgaccgtggacaagtctagcagcaccgcctacatgcagctgagcagccctacaagcgaggacagcgccgtgtattattgcacccggtcttggcggggcaacagcttcgattattggggccagggcacaaccctgaccgtgtctagcaccaccaccgactacaaggacgacgacgacaagcccgctcctagacctcctacaccagctcctacaatcgccagccagcctctgtctctgaggccagaagcttgtagacctgctgctggcggagccgtgcatacaagaggactggatttcgcctgcgacttctgggtgctcgtggttgttggcggagtgctggcctgttactctctgctggtcaccgtggccttcatcatcttttgggtccgaagcaagcggagccggctgctgcacagcgactacatgaacatgacccctagacggcccggacctaccagaaagcactaccagccttacgctcctcctagagacttcgccgcctaccggtccagagtgaagttcagcagatccgctgatgcccctgcctatcagcagggccagaaccagctgtacaacgagctgaacctggggagaagagaagagtacgacgtgctggacaagcggagaggcagagatcctgagatgggcggcaagcccagacggaagaatcctcaagagggcctgtacaatgaactgcagaaagacaagatggccgaggcctacagcgagatcggaatgaagggcgagcgcagaagaggcaagggacacgatggactgtaccagggcctgagcaccgccaccaaggatacctatgatgccctgcacatgcaggccctgcctccaagataa

SEQ ID NO: 47 - DNA, 2034 bp, synthetic construct
  source 1..2034: mol_type = other DNA
atggctctgcctgtgacagctctgctgctgcctctggctctgcttctgcatgccgccagaccgcaagtgcagctcgtggaaagcggcggcgggctcgtgcaagccggggggagcctgagactggcctgcaccgctagcggcaacatcttcgctagccaagtgatgaactggtacagacaagcccccggcagccctagagagctggtggccaccatcacccccggcggcagaaccacctacgccgacagcgccaagggcagattcaccgtggccaccgacaacgccaaggccaccgcctacctgcagctgacaagcctgctggaggccgaggacaccggcatctactactgcgcccccgctagatacgccgcctgcagcgccctggacgtgaagctgagcttcacaagctggggccaaggcacccaagtgaccgtgagcagcggaagcactagcggaagcggaaagccaggaagcggagaaggaagcactaagggacaagtgcagctggtcgagagcggcgggggcctcgtccaacccggcggcagcctgagactgagctgcgccgctagcggcttcaccttcagcagctacgccatgggctgggctagacaagtgcccggcaaggacgtggagtgggtgagcggcatctacagcgacggcagcacctactacgccgacagcgtgaagggcagattcaccatcagcagatacaacgccaagaacaccgtgtacctgcagatgaacagcctgaagcccgaggacaccgccgtgtactactgcgccaccgatcctaccctcgagaatcagacaaccgcctggggccaagggacccaagtgaccgtgagcagcgccgaggatctggccgtgtactactgccagaacgactacagctaccccttcacctttggcagcggcaccaagctggaaatcaaaggcggaggcggatctggcggcggaggtagcggtggcggaggatctcaagttcagctgcaacagcctggcgccgaactcgttagacctggcgcttctgtgaagctgtcctgcaaggccagcggctacacctttaccagctactggatcaactgggtcaagcagaggccaggccagggcctcgaatggatcggcaatatctaccccagcgacagctacaccaactacaatcagaagttcaaggacaaggccacactgaccgtggacaagtctagcagcaccgcctacatgcagctgagcagccctacaagcgaggacagcgccgtgtattattgcacccggtcttggcggggcaacagcttcgattattggggccagggcacaaccctgaccgtgtctagcaccaccaccgactacaaggacgacgacgacaagcccgctcctagacctcctacaccagctcctacaatcgccagccagcctctgtctctgaggccagaagcttgtagacctgctgctggcggagccgtgcatacaagaggactggatttcgcctgcgacttctgggtgctcgtggttgttggcggagtgctggcctgttactctctgctggtcaccgtggccttcatcatcttttgggtccgaagcaagcggagccggctgctgcacagcgactacatgaacatgacccctagacggcccggacctaccagaaagcactaccagccttacgctcctcctagagacttcgccgcctaccggtccagagtgaagttcagcagatccgctgatgcccctgcctatcagcagggccagaaccagctgtacaacgagctgaacctggggagaagagaagagtacgacgtgctggacaagcggagaggcagagatcctgagatgggcggcaagcccagacggaagaatcctcaagagggcctgtacaatgaactgcagaaagacaagatggccgaggcctacagcgagatcggaatgaagggcgagcgcagaagaggcaagggacacgatggactgtaccagggcctgagcaccgccaccaaggatacctatgatgccctgcacatgcaggccctgcctccaagataa

SEQ ID NO: 48 - DNA, 2820 bp, synthetic construct
  source 1..2820: mol_type = other DNA
caatggctctgcctgtgacagctctgctgctgcctctggctctgcttctgcatgccgccagaccgcaagtgcaactcgtcgaaagcggcggcgggctcgtgcaacctggggggagcctgagactgagctgcaccgctagcggcttcagactggactactacgccatcggctggttcagacaagcccccggcaaggagagagaggccatcagctgcatcgacatcaccggcatgcacaccaactacggcgacagcgtgatgggcagattcaccatcagcagagacgacgccaagagaaccgtgtacctgcagatgaacagcctggaggccgaggacaccggcatctactactgcgcccccgctcagtacgccgcctgcagcgccctgggcgtgaaggtgagcttcacaagctggggccaaggcacccaagtgaccgtgagccccggaagcactagcggaagcggaaagccaggaagcggagaaggaagcactaagggacaagtgcaactcgtggagagcgggggggggctggtgcagcccggggggagcctgagactgagctgcgccgctagcggcttcaccttcagcagctacgccatgggctgggctagacaagtgcccggcaaagaggtggagtgggtgagcggcatctacagcgacggcagcaccaactacgccgacagcgtgaagggcagattcaccatcagcagagacaacgccaagaacaccgtgtacctgcagatgaacagcctgagacccgaggacaccgccgtgtaccactgcgccacagatcccacagtgcacagcgatctgcccgtctgggggcaaggcaccctggtcaccgtgagcagcgccgaggatctggccgtgtactactgccagaacgactacagctaccccttcacctttggcagcggcaccaagctggaaatcaaaggcggaggcggatctggcggcggaggtagcggtggcggaggatctcaagttcagctgcaacagcctggcgccgaactcgttagacctggcgcttctgtgaagctgtcctgcaaggccagcggctacacctttaccagctactggatcaactgggtcaagcagaggccaggccagggcctcgaatggatcggcaatatctaccccagcgacagctacaccaactacaatcagaagttcaaggacaaggccacactgaccgtggacaagtctagcagcaccgcctacatgcagctgagcagccctacaagcgaggacagcgccgtgtattattgcacccggtcttggcggggcaacagcttcgattattggggccagggcacaaccctgaccgtgtctagcaccaccaccgactacaaggacgacgacgacaagcccgctcctagacctcctacaccagctcctacaatcgccagccagcctctgtctctgaggccagaagcttgtagacctgctgctggcggagccgtgcatacaagaggactggatttcgcctgcgacttctgggtgctcgtggttgttggcggagtgctggcctgttactctctgctggtcaccgtggccttcatcatcttttgggtccgaagcaagcggagccggctgctgcacagcgactacatgaacatgacccctagacggcccggacctaccagaaagcactaccagccttacgctcctcctagagacttcgccgcctaccggtccagagtgaagttcagcagatccgctgatgcccctgcctatcagcagggccagaaccagctgtacaacgagctgaacctggggagaagagaagagtacgacgtgctggacaagcggagaggcagagatcctgagatgggcggcaagcccagacggaagaatcctcaagagggcctgtacaatgaactgcagaaagacaagatggccgaggcctacagcgagatcggaatgaagggcgagcgcagaagaggcaagggacacgatggactgtaccagggcctgagcaccgccaccaaggatacctatgatgccctgcacatgcaggccctgcctccaagataaagtgcaactcgtcgaaagcggcggcgggctcgtgcaacctggggggagcctgagactgagctgcaccgctagcggcttcagactggactactacgccatcggctggttcagacaagcccccggcaaggagagagaggccatcagctgcatcgacatcaccggcatgcacaccaactacggcgacagcgtgatgggcagattcaccatcagcagagacgacgccaagagaaccgtgtacctgcagatgaacagcctggaggccgaggacaccggcatctactactgcgcccccgctcagtacgccgcctgcagcgccctgggcgtgaaggtgagcttcacaagctggggccaaggcacccaagtgaccgtgagccccggaagcactagcggaagcggaaagccaggaagcggagaaggaagcactaagggacaagtgcaactcgtggagagcgggggggggctggtgcagcccggggggagcctgagactgagctgcgccgctagcggcttcaccttcagcagctacgccatgggctgggctagacaagtgcccggcaaagaggtggagtgggtgagcggcatctacagcgacggcagcaccaactacgccgacagcgtgaagggcagattcaccatcagcagagacaacgccaagaacaccgtgtacctgcagatgaacagcctgagacccgaggacaccgccgtgtaccactgcgccacagatcccacagtgcacagcgatctgcccgtctgggggcaaggcaccctggtcaccgtgagcagc

SEQ ID NO: 49 - DNA, 2034 bp, synthetic construct
  source 1..2034: mol_type = other DNA
atggctctgcctgtgacagctctgctgctgcctctggctctgcttctgcatgccgccagaccgcaagtgcaactcgtcgaaagcggcggcgggctcgtgcaacctggggggagcctgagactgagctgcaccgctagcggcttcagactggactactacgccatcggctggttcagacaagcccccggcaaggagagagaggccatcagctgcatcgacatcaccggcatgcacaccaactacggcgacagcgtgatgggcagattcaccatcagcagagacgacgccaagagaaccgtgtacctgcagatgaacagcctggaggccgaggacaccggcatctactactgcgcccccgctcagtacgccgcctgcagcgccctgggcgtgaaggtgagcttcacaagctggggccaaggcacccaagtgaccgtgagccccggaagcactagcggaagcggaaagccaggaagcggagaaggaagcactaagggacaagtgcagctggtcgagagcggcgggggcctcgtccaacccggcggcagcctgagactgagctgcgccgctagcggcttcaccttcagcagctacgccatgggctgggctagacaagtgcccggcaaggacgtggagtgggtgagcggcatctacagcgacggcagcacctactacgccgacagcgtgaagggcagattcaccatcagcagatacaacgccaagaacaccgtgtacctgcagatgaacagcctgaagcccgaggacaccgccgtgtactactgcgccaccgatcctaccctcgagaatcagacaaccgcctggggccaagggacccaagtgaccgtgagcagcgccgaggatctggccgtgtactactgccagaacgactacagctaccccttcacctttggcagcggcaccaagctggaaatcaaaggcggaggcggatctggcggcggaggtagcggtggcggaggatctcaagttcagctgcaacagcctggcgccgaactcgttagacctggcgcttctgtgaagctgtcctgcaaggccagcggctacacctttaccagctactggatcaactgggtcaagcagaggccaggccagggcctcgaatggatcggcaatatctaccccagcgacagctacaccaactacaatcagaagttcaaggacaaggccacactgaccgtggacaagtctagcagcaccgcctacatgcagctgagcagccctacaagcgaggacagcgccgtgtattattgcacccggtcttggcggggcaacagcttcgattattggggccagggcacaaccctgaccgtgtctagcaccaccaccgactacaaggacgacgacgacaagcccgctcctagacctcctacaccagctcctacaatcgccagccagcctctgtctctgaggccagaagcttgtagacctgctgctggcggagccgtgcatacaagaggactggatttcgcctgcgacttctgggtgctcgtggttgttggcggagtgctggcctgttactctctgctggtcaccgtggccttcatcatcttttgggtccgaagcaagcggagccggctgctgcacagcgactacatgaacatgacccctagacggcccggacctaccagaaagcactaccagccttacgctcctcctagagacttcgccgcctaccggtccagagtgaagttcagcagatccgctgatgcccctgcctatcagcagggccagaaccagctgtacaacgagctgaacctggggagaagagaagagtacgacgtgctggacaagcggagaggcagagatcctgagatgggcggcaagcccagacggaagaatcctcaagagggcctgtacaatgaactgcagaaagacaagatggccgaggcctacagcgagatcggaatgaagggcgagcgcagaagaggcaagggacacgatggactgtaccagggcctgagcaccgccaccaaggatacctatgatgccctgcacatgcaggccctgcctccaagataa

SEQ ID NO: 50 - DNA, 2034 bp, synthetic construct
  source 1..2034: mol_type = other DNA
atggctctgcctgtgacagctctgctgctgcctctggctctgcttctgcatgccgccagaccgcaagtgcaactcgtcgaaagcggcggcgggctcgtgcaacctggggggagcctgagactgagctgcaccgctagcggcttcagactggactactacgccatcggctggttcagacaagcccccggcaaggagagagaggccatcgcctgcatcgacatcaccggcttccacaccaactacggcgacagcgtgagcggcagattcaccatcagcagagacaacgccggcaccaccgtgtacctgcagatgaacagcctggaggccgaggacaccggcatctactactgcgcccccgctagatacgccgcctgcagcgccctggacgtgaagctgagcttcacaagctggggccaaggcacccaagtgaccgtgagcagcggaagcactagcggaagcggaaagccaggaagcggagaaggaagcactaagggacaagtgcaactcgtggagagcgggggggggctggtgcagcccggggggagcctgagactgagctgcgccgctagcggcttcaccttcagcagctacgccatgggctgggctagacaagtgcccggcaaagaggtggagtgggtgagcggcatctacagcgacggcagcaccaactacgccgacagcgtgaagggcagattcaccatcagcagagacaacgccaagaacaccgtgtacctgcagatgaacagcctgagacccgaggacaccgccgtgtaccactgcgccacagatcccacagtgcacagcgatctgcccgtctgggggcaaggcaccctggtcaccgtgagcagcgccgaggatctggccgtgtactactgccagaacgactacagctaccccttcacctttggcagcggcaccaagctggaaatcaaaggcggaggcggatctggcggcggaggtagcggtggcggaggatctcaagttcagctgcaacagcctggcgccgaactcgttagacctggcgcttctgtgaagctgtcctgcaaggccagcggctacacctttaccagctactggatcaactgggtcaagcagaggccaggccagggcctcgaatggatcggcaatatctaccccagcgacagctacaccaactacaatcagaagttcaaggacaaggccacactgaccgtggacaagtctagcagcaccgcctacatgcagctgagcagccctacaagcgaggacagcgccgtgtattattgcacccggtcttggcggggcaacagcttcgattattggggccagggcacaaccctgaccgtgtctagcaccaccaccgactacaaggacgacgacgacaagcccgctcctagacctcctacaccagctcctacaatcgccagccagcctctgtctctgaggccagaagcttgtagacctgctgctggcggagccgtgcatacaagaggactggatttcgcctgcgacttctgggtgctcgtggttgttggcggagtgctggcctgttactctctgctggtcaccgtggccttcatcatcttttgggtccgaagcaagcggagccggctgctgcacagcgactacatgaacatgacccctagacggcccggacctaccagaaagcactaccagccttacgctcctcctagagacttcgccgcctaccggtccagagtgaagttcagcagatccgctgatgcccctgcctatcagcagggccagaaccagctgtacaacgagctgaacctggggagaagagaagagtacgacgtgctggacaagcggagaggcagagatcctgagatgggcggcaagcccagacggaagaatcctcaagagggcctgtacaatgaactgcagaaagacaagatggccgaggcctacagcgagatcggaatgaagggcgagcgcagaagaggcaagggacacgatggactgtaccagggcctgagcaccgccaccaaggatacctatgatgccctgcacatgcaggccctgcctccaagataa

SEQ ID NO: 51 - DNA, 2034 bp, synthetic construct
  source 1..2034: mol_type = other DNA
atggctctgcctgtgacagctctgctgctgcctctggctctgcttctgcatgccgccagaccgcaagtgcaactcgtcgaaagcggcggcgggctcgtgcaacctggggggagcctgagactgagctgcaccgctagcggcttcagactggactactacgccatcggctggttcagacaagcccccggcaaggagagagaggccatcgcctgcatcgacatcaccggcttccacaccaactacggcgacagcgtgagcggcagattcaccatcagcagagacaacgccggcaccaccgtgtacctgcagatgaacagcctggaggccgaggacaccggcatctactactgcgcccccgctagatacgccgcctgcagcgccctggacgtgaagctgagcttcacaagctggggccaaggcacccaagtgaccgtgagcagcggaagcactagcggaagcggaaagccaggaagcggagaaggaagcactaagggacaagtgcagctggtcgagagcggcgggggcctcgtccaacccggcggcagcctgagactgagctgcgccgctagcggcttcaccttcagcagctacgccatgggctgggctagacaagtgcccggcaaggacgtggagtgggtgagcggcatctacagcgacggcagcacctactacgccgacagcgtgaagggcagattcaccatcagcagatacaacgccaagaacaccgtgtacctgcagatgaacagcctgaagcccgaggacaccgccgtgtactactgcgccaccgatcctaccctcgagaatcagacaaccgcctggggccaagggacccaagtgaccgtgagcagcgccgaggatctggccgtgtactactgccagaacgactacagctaccccttcacctttggcagcggcaccaagctggaaatcaaaggcggaggcggatctggcggcggaggtagcggtggcggaggatctcaagttcagctgcaacagcctggcgccgaactcgttagacctggcgcttctgtgaagctgtcctgcaaggccagcggctacacctttaccagctactggatcaactgggtcaagcagaggccaggccagggcctcgaatggatcggcaatatctaccccagcgacagctacaccaactacaatcagaagttcaaggacaaggccacactgaccgtggacaagtctagcagcaccgcctacatgcagctgagcagccctacaagcgaggacagcgccgtgtattattgcacccggtcttggcggggcaacagcttcgattattggggccagggcacaaccctgaccgtgtctagcaccaccaccgactacaaggacgacgacgacaagcccgctcctagacctcctacaccagctcctacaatcgccagccagcctctgtctctgaggccagaagcttgtagacctgctgctggcggagccgtgcatacaagaggactggatttcgcctgcgacttctgggtgctcgtggttgttggcggagtgctggcctgttactctctgctggtcaccgtggccttcatcatcttttgggtccgaagcaagcggagccggctgctgcacagcgactacatgaacatgacccctagacggcccggacctaccagaaagcactaccagccttacgctcctcctagagacttcgccgcctaccggtccagagtgaagttcagcagatccgctgatgcccctgcctatcagcagggccagaaccagctgtacaacgagctgaacctggggagaagagaagagtacgacgtgctggacaagcggagaggcagagatcctgagatgggcggcaagcccagacggaagaatcctcaagagggcctgtacaatgaactgcagaaagacaagatggccgaggcctacagcgagatcggaatgaagggcgagcgcagaagaggcaagggacacgatggactgtaccagggcctgagcaccgccaccaaggatacctatgatgccctgcacatgcaggccctgcctccaagataa